European Patent Application EP 4 768 587 A1, published July 1, 2026. Title: 抑制淀粉样前体蛋白（APP）基因表达的siRNA、药物及其应用. Applicant: 广州必贝特医药股份有限公司. Application CN. The sequence listing filed with the application follows.

SEQUENCE LISTING (186 sequences)

SEQ ID NO: 1 - RNA, 21 nt, synthetic construct
  source 1..21: mol_type = other RNA
ggcagaacggctacgaaaata

SEQ ID NO: 2 - RNA, 21 nt, synthetic construct
  source 1..21: mol_type = other RNA
tattttcgtagccgttctgcc

SEQ ID NO: 3 - RNA, 21 nt, synthetic construct
  source 1..21: mol_type = other RNA
ggcagaacggctacgaaaata

SEQ ID NO: 4 - RNA, 23 nt, synthetic construct
  source 1..23: mol_type = other RNA
tattttcgtagccgttctgctgc

SEQ ID NO: 5 - RNA, 19 nt, synthetic construct
  source 1..19: mol_type = other RNA
gcctacaagttctttgaga

SEQ ID NO: 6 - RNA, 21 nt, synthetic construct
  source 1..21: mol_type = other RNA
tctcaaagaacttgtaggctg

SEQ ID NO: 7 - RNA, 19 nt, synthetic construct
  source 1..19: mol_type = other RNA
cccacaagttctttgagca

SEQ ID NO: 8 - RNA, 21 nt, synthetic construct
  source 1..21: mol_type = other RNA
tgctcaaagaacttgtcggtt

SEQ ID NO: 9 - RNA, 19 nt, synthetic construct
  source 1..19: mol_type = other RNA
cacaagttctttgagcaga

SEQ ID NO: 10 - RNA, 21 nt, synthetic construct
  source 1..21: mol_type = other RNA
tctgctcaaagaacttgtggg

SEQ ID NO: 11 - RNA, 21 nt, synthetic construct
  source 1..21: mol_type = other RNA
cacaagttctttgagcagata

SEQ ID NO: 12 - RNA, 21 nt, synthetic construct
  source 1..21: mol_type = other RNA
tatctgctcaaagaacttgtg

SEQ ID NO: 13 - RNA, 21 nt, synthetic construct
  source 1..21: mol_type = other RNA
cacaagttctttgagcaaata

SEQ ID NO: 14 - RNA, 21 nt, synthetic construct
  source 1..21: mol_type = other RNA
tatttgctcaaagaacttgtg

SEQ ID NO: 15 - RNA, 21 nt, synthetic construct
  source 1..21: mol_type = other RNA
ccacaagttctttgagcagaa

SEQ ID NO: 16 - RNA, 21 nt, synthetic construct
  source 1..21: mol_type = other RNA
ttctgctcaaagaacttgtgg

SEQ ID NO: 17 - RNA, 21 nt, synthetic construct
  source 1..21: mol_type = other RNA
ctatgagcgcatgaatcagta

SEQ ID NO: 18 - RNA, 21 nt, synthetic construct
  source 1..21: mol_type = other RNA
tactgattcatgcgctcatag

SEQ ID NO: 19 - RNA, 21 nt, synthetic construct
  source 1..21: mol_type = other RNA
gccgtgtgatttatgagcgca

SEQ ID NO: 20 - RNA, 21 nt, synthetic construct
  source 1..21: mol_type = other RNA
tgcgctcataaatcacacggc

SEQ ID NO: 21 - RNA, 21 nt, synthetic construct
  source 1..21: mol_type = other RNA
ccccgtgtgatttatgagcga

SEQ ID NO: 22 - RNA, 23 nt, synthetic construct
  source 1..23: mol_type = other RNA
tcgctcataaatcacacgggggt

SEQ ID NO: 23 - RNA, 21 nt, synthetic construct
  source 1..21: mol_type = other RNA
catgacacacctccgtgtgaa

SEQ ID NO: 24 - RNA, 21 nt, synthetic construct
  source 1..21: mol_type = other RNA
ttcacacggaggtgtgtcatg

SEQ ID NO: 25 - RNA, 21 nt, synthetic construct
  source 1..21: mol_type = other RNA
ccgtaaagaatttagctgtaa

SEQ ID NO: 26 - RNA, 21 nt, synthetic construct
  source 1..21: mol_type = other RNA
ttacagctaaattctttacgg

SEQ ID NO: 27 - RNA, 21 nt, synthetic construct
  source 1..21: mol_type = other RNA
cgggttttgtgtactgtaaaa

SEQ ID NO: 28 - RNA, 21 nt, synthetic construct
  source 1..21: mol_type = other RNA
ttttacagtacacaaaacccg

SEQ ID NO: 29 - RNA, 21 nt, synthetic construct
  source 1..21: mol_type = other RNA
catccagcatttccaggagaa

SEQ ID NO: 30 - RNA, 23 nt, synthetic construct
  source 1..23: mol_type = other RNA
ttctcctggaaatgctggatgac

SEQ ID NO: 31 - RNA, 21 nt, synthetic construct
  source 1..21: mol_type = other RNA
ctatccagcatttccaggaga

SEQ ID NO: 32 - RNA, 23 nt, synthetic construct
  source 1..23: mol_type = other RNA
tctcctggaaatgctggatagct

SEQ ID NO: 33 - RNA, 21 nt, synthetic construct
  source 1..21: mol_type = other RNA
catcaaactagtgcatgaata

SEQ ID NO: 34 - RNA, 21 nt, synthetic construct
  source 1..21: mol_type = other RNA
tattcatgcactagtttgatg

SEQ ID NO: 35 - RNA, 21 nt, synthetic construct
  source 1..21: mol_type = other RNA
ccgtatcaaactagtgcatga

SEQ ID NO: 36 - RNA, 21 nt, synthetic construct
  source 1..21: mol_type = other RNA
tcatgcactagtttgatacgg

SEQ ID NO: 37 - RNA, 21 nt, synthetic construct
  source 1..21: mol_type = other RNA
cggtgagtttgtaagtgatga

SEQ ID NO: 38 - RNA, 21 nt, synthetic construct
  source 1..21: mol_type = other RNA
tcatcacttacaaactcaccg

SEQ ID NO: 39 - RNA, 21 nt, synthetic construct
  source 1..21: mol_type = other RNA
cagtttgtaagtgatgcccta

SEQ ID NO: 40 - RNA, 21 nt, synthetic construct
  source 1..21: mol_type = other RNA
tagggcatcacttacaaactg

SEQ ID NO: 41 - RNA, 21 nt, synthetic construct
  source 1..21: mol_type = other RNA
cgcttagttggtgagtttgta

SEQ ID NO: 42 - RNA, 21 nt, synthetic construct
  source 1..21: mol_type = other RNA
tacaaactcaccaactaagcg

SEQ ID NO: 43 - RNA, 21 nt, synthetic construct
  source 1..21: mol_type = other RNA
gggatatgaagttcatcatca

SEQ ID NO: 44 - RNA, 21 nt, synthetic construct
  source 1..21: mol_type = other RNA
tgatgatgaacttcatatccc

SEQ ID NO: 45 - RNA, 20 nt, synthetic construct
  source 1..20: mol_type = other RNA
acgactcaggatatgaagtt

SEQ ID NO: 46 - RNA, 21 nt, synthetic construct
  source 1..21: mol_type = other RNA
taacttcatatcctgagtcgt

SEQ ID NO: 47 - RNA, 21 nt, synthetic construct
  source 1..21: mol_type = other RNA
cgaactgcagatcaccaatga

SEQ ID NO: 48 - RNA, 21 nt, synthetic construct
  source 1..21: mol_type = other RNA
tcattggtgatctgcagttcg

SEQ ID NO: 49 - RNA, 21 nt, synthetic construct
  source 1..21: mol_type = other RNA
ctaccctgaactgcagatcaa

SEQ ID NO: 50 - RNA, 23 nt, synthetic construct
  source 1..23: mol_type = other RNA
ttgatctgcagttcagggtaggc

SEQ ID NO: 51 - RNA, 21 nt, synthetic construct
  source 1..21: mol_type = other RNA
gaagtctaccctgaactgcaa

SEQ ID NO: 52 - RNA, 23 nt, synthetic construct
  source 1..23: mol_type = other RNA
ttgcagttcagggtagacttctt

SEQ ID NO: 53 - RNA, 21 nt, synthetic construct
  source 1..21: mol_type = other RNA
caggtacccactgatggtaaa

SEQ ID NO: 54 - RNA, 21 nt, synthetic construct
  source 1..21: mol_type = other RNA
tttaccatcagtgggtacctg

SEQ ID NO: 55 - RNA, 21 nt, synthetic construct
  source 1..21: mol_type = other RNA
gcacccactgatggtaatgca

SEQ ID NO: 56 - RNA, 21 nt, synthetic construct
  source 1..21: mol_type = other RNA
tgcattaccatcagtgggtgc

SEQ ID NO: 57 - RNA, 21 nt, synthetic construct
  source 1..21: mol_type = other RNA
gccagtgaccatccagaacta

SEQ ID NO: 58 - RNA, 23 nt, synthetic construct
  source 1..23: mol_type = other RNA
tagttctggatggtcactggctg

SEQ ID NO: 59 - RNA, 21 nt, synthetic construct
  source 1..21: mol_type = other RNA
gggagtgggattcagatccaa

SEQ ID NO: 60 - RNA, 21 nt, synthetic construct
  source 1..21: mol_type = other RNA
ttggatctgaatcccactccc

SEQ ID NO: 61 - RNA, 21 nt, synthetic construct
  source 1..21: mol_type = other RNA
cccgacatgactcaggatata

SEQ ID NO: 62 - RNA, 21 nt, synthetic construct
  source 1..21: mol_type = other RNA
tatatcctgagtcatgtcggg

SEQ ID NO: 63 - RNA, 21 nt, synthetic construct
  source 1..21: mol_type = other RNA
cagtaccaacttgcatgacta

SEQ ID NO: 64 - RNA, 21 nt, synthetic construct
  source 1..21: mol_type = other RNA
tagtcatgcaagttggtactg

SEQ ID NO: 65 - RNA, 21 nt, synthetic construct
  source 1..21: mol_type = other RNA
ggtgagaagagtaccaactta

SEQ ID NO: 66 - RNA, 21 nt, synthetic construct
  source 1..21: mol_type = other RNA
taagttggtactcttctcacc

SEQ ID NO: 67 - RNA, 21 nt, synthetic construct
  source 1..21: mol_type = other RNA
cagacatgcagtgagaagaga

SEQ ID NO: 68 - RNA, 21 nt, synthetic construct
  source 1..21: mol_type = other RNA
tctcttctcactgcatgtctg

SEQ ID NO: 69 - RNA, 19 nt, synthetic construct
  source 1..19: mol_type = other RNA
tatgcccatttccagaaaa

SEQ ID NO: 70 - RNA, 21 nt, synthetic construct
  source 1..21: mol_type = other RNA
ttttctggaaatgggcatgtt

SEQ ID NO: 71 - RNA, 21 nt, synthetic construct
  source 1..21: mol_type = other RNA
gcgaagatggatgcagaatta

SEQ ID NO: 72 - RNA, 21 nt, synthetic construct
  source 1..21: mol_type = other RNA
taattctgcatccatcttcgc

SEQ ID NO: 73 - RNA, 21 nt, synthetic construct
  source 1..21: mol_type = other RNA
cgaagtgaagatggatgcaga

SEQ ID NO: 74 - RNA, 21 nt, synthetic construct
  source 1..21: mol_type = other RNA
tctgcatccatcttcacttcg

SEQ ID NO: 75 - RNA, 21 nt, synthetic construct
  source 1..21: mol_type = other RNA
gctgtccaagatgcagcagaa

SEQ ID NO: 76 - RNA, 21 nt, synthetic construct
  source 1..21: mol_type = other RNA
ttctgctgcatcttggacagc

SEQ ID NO: 77 - RNA, 21 nt, synthetic construct
  source 1..21: mol_type = other RNA
gaacctacaagttctttgaga

SEQ ID NO: 78 - RNA, 21 nt, synthetic construct
  source 1..21: mol_type = other RNA
tctcaaagaacttgtaggttc

SEQ ID NO: 79 - RNA, 21 nt, synthetic construct
  source 1..21: mol_type = other RNA
gacctacaagttctttgagca

SEQ ID NO: 80 - RNA, 21 nt, synthetic construct
  source 1..21: mol_type = other RNA
tgctcaaagaacttgtaggtc

SEQ ID NO: 81 - RNA, 21 nt, synthetic construct
  source 1..21: mol_type = other RNA
cccacaagttctttgagcaga

SEQ ID NO: 82 - RNA, 21 nt, synthetic construct
  source 1..21: mol_type = other RNA
tctgctcaaagaacttgtggg

SEQ ID NO: 83 - RNA, 21 nt, synthetic construct
  source 1..21: mol_type = other RNA
gaaatccaacctacaagttca

SEQ ID NO: 84 - RNA, 21 nt, synthetic construct
  source 1..21: mol_type = other RNA
tgaacttgtaggttggatttc

SEQ ID NO: 85 - RNA, 21 nt, synthetic construct
  source 1..21: mol_type = other RNA
gcaggagaaagtggaatctta

SEQ ID NO: 86 - RNA, 21 nt, synthetic construct
  source 1..21: mol_type = other RNA
taagattccactttctcctgc

SEQ ID NO: 87 - RNA, 21 nt, synthetic construct
  source 1..21: mol_type = other RNA
cactcaggatatgaagttcaa

SEQ ID NO: 88 - RNA, 21 nt, synthetic construct
  source 1..21: mol_type = other RNA
ttgaacttcatatcctgagtg

SEQ ID NO: 89 - RNA, 21 nt, synthetic construct
  source 1..21: mol_type = other RNA
ccaccctgaactgcagatcaa

SEQ ID NO: 90 - RNA, 21 nt, synthetic construct
  source 1..21: mol_type = other RNA
ttgatctgcagttcagggtgg

SEQ ID NO: 91 - RNA, 21 nt, synthetic construct
  source 1..21: mol_type = other RNA
gaccaatgtggtagaagccaa

SEQ ID NO: 92 - RNA, 21 nt, synthetic construct
  source 1..21: mol_type = other RNA
ttggcttctaccacattggtc

SEQ ID NO: 93 - RNA, 21 nt, synthetic construct
  source 1..21: mol_type = other RNA
gtgcacatgaatgtccagaaa

SEQ ID NO: 94 - RNA, 21 nt, synthetic construct
  source 1..21: mol_type = other RNA
tttctggacattcatgtgcac

SEQ ID NO: 95 - RNA, 21 nt, synthetic construct
  source 1..21: mol_type = other RNA
ccgccaagaagtctaccctga

SEQ ID NO: 96 - RNA, 21 nt, synthetic construct
  source 1..21: mol_type = other RNA
tcagggtagacttcttggcgg

SEQ ID NO: 97 - RNA, 21 nt, synthetic construct
  source 1..21: mol_type = other RNA
gagcaaagaacttgcctaaaa

SEQ ID NO: 98 - RNA, 21 nt, synthetic construct
  source 1..21: mol_type = other RNA
ttttaggcaagttctttgctc

SEQ ID NO: 99 - RNA, 21 nt, synthetic construct
  source 1..21: mol_type = other RNA
caagaaggcagttatccagca

SEQ ID NO: 100 - RNA, 21 nt, synthetic construct
  source 1..21: mol_type = other RNA
tgctggataactgccttcttg

SEQ ID NO: 101 - RNA, 21 nt, synthetic construct
  source 1..21: mol_type = other RNA
gctcaatatgctaaagaagta

SEQ ID NO: 102 - RNA, 21 nt, synthetic construct
  source 1..21: mol_type = other RNA
tacttctttagcatattgagc

SEQ ID NO: 103 - RNA, 21 nt, synthetic construct
  source 1..21: mol_type = other RNA
gagagcaaaactattcagata

SEQ ID NO: 104 - RNA, 21 nt, synthetic construct
  source 1..21: mol_type = other RNA
tatctgaatagttttgctctc

SEQ ID NO: 105 - RNA, 21 nt, synthetic construct
  source 1..21: mol_type = other RNA
cgatgagctgcttcagaaaga

SEQ ID NO: 106 - RNA, 21 nt, synthetic construct
  source 1..21: mol_type = other RNA
tctttctgaagcagctcatcg

SEQ ID NO: 107 - RNA, 21 nt, synthetic construct
  source 1..21: mol_type = other RNA
ggcaaaactattcagatgaca

SEQ ID NO: 108 - RNA, 21 nt, synthetic construct
  source 1..21: mol_type = other RNA
tgtcatctgaatagttttgcc

SEQ ID NO: 109 - RNA, 21 nt, synthetic construct
  source 1..21: mol_type = other RNA
cacggaaacgatgctctcata

SEQ ID NO: 110 - RNA, 21 nt, synthetic construct
  source 1..21: mol_type = other RNA
tatgagagcatcgtttccgtg

SEQ ID NO: 111 - RNA, 21 nt, synthetic construct
  source 1..21: mol_type = other RNA
ccctcatgccatctttgacca

SEQ ID NO: 112 - RNA, 21 nt, synthetic construct
  source 1..21: mol_type = other RNA
tggtcaaagatggcatgaggg

SEQ ID NO: 113 - RNA, 21 nt, synthetic construct
  source 1..21: mol_type = other RNA
ggatgctctcatgccatctta

SEQ ID NO: 114 - RNA, 21 nt, synthetic construct
  source 1..21: mol_type = other RNA
taagatggcatgagagcatcc

SEQ ID NO: 115 - RNA, 21 nt, synthetic construct
  source 1..21: mol_type = other RNA
gggttctgggttgacaaataa

SEQ ID NO: 116 - RNA, 21 nt, synthetic construct
  source 1..21: mol_type = other RNA
ttatttgtcaacccagaaccc

SEQ ID NO: 117 - RNA, 21 nt, synthetic construct
  source 1..21: mol_type = other RNA
cgatatgaagttcatcatcaa

SEQ ID NO: 118 - RNA, 21 nt, synthetic construct
  source 1..21: mol_type = other RNA
ttgatgatgaacttcatatcg

SEQ ID NO: 119 - RNA, 21 nt, synthetic construct
  source 1..21: mol_type = other RNA
ggagttcatcatcaaaaatta

SEQ ID NO: 120 - RNA, 21 nt, synthetic construct
  source 1..21: mol_type = other RNA
taatttttgatgatgaactcc

SEQ ID NO: 121 - RNA, 21 nt, synthetic construct
  source 1..21: mol_type = other RNA
gtcatcaaaaattggtgttca

SEQ ID NO: 122 - RNA, 21 nt, synthetic construct
  source 1..21: mol_type = other RNA
tgaacaccaatttttgatgac

SEQ ID NO: 123 - RNA, 21 nt, synthetic construct
  source 1..21: mol_type = other RNA
ccatcaaaaattggtgttcta

SEQ ID NO: 124 - RNA, 21 nt, synthetic construct
  source 1..21: mol_type = other RNA
tagaacaccaatttttgatgg

SEQ ID NO: 125 - RNA, 21 nt, synthetic construct
  source 1..21: mol_type = other RNA
gatgggttttgtgtactgtaa

SEQ ID NO: 126 - RNA, 21 nt, synthetic construct
  source 1..21: mol_type = other RNA
ttacagtacacaaaacccatc

SEQ ID NO: 127 - RNA, 21 nt, synthetic construct
  source 1..21: mol_type = other RNA
ctaatgggttttgtgtactga

SEQ ID NO: 128 - RNA, 21 nt, synthetic construct
  source 1..21: mol_type = other RNA
tcagtacacaaaacccattag

SEQ ID NO: 129 - RNA, 21 nt, synthetic construct
  source 1..21: mol_type = other RNA
cattaatgggttttgtgtaca

SEQ ID NO: 130 - RNA, 21 nt, synthetic construct
  source 1..21: mol_type = other RNA
tgtacacaaaacccattaatg

SEQ ID NO: 131 - RNA, 21 nt, synthetic construct
  source 1..21: mol_type = other RNA
ctattaatgggttttgtgtaa

SEQ ID NO: 132 - RNA, 21 nt, synthetic construct
  source 1..21: mol_type = other RNA
ttacacaaaacccattaatag

SEQ ID NO: 133 - RNA, 21 nt, synthetic construct
  source 1..21: mol_type = other RNA
cacattattaatgggttttga

SEQ ID NO: 134 - RNA, 21 nt, synthetic construct
  source 1..21: mol_type = other RNA
tcaaaacccattaataatgtg

SEQ ID NO: 135 - RNA, 21 nt, synthetic construct
  source 1..21: mol_type = other RNA
cgtaaagaatttagctgtata

SEQ ID NO: 136 - RNA, 21 nt, synthetic construct
  source 1..21: mol_type = other RNA
tatacagctaaattctttacg

SEQ ID NO: 137 - RNA, 21 nt, synthetic construct
  source 1..21: mol_type = other RNA
cgaatagattctctcctgata

SEQ ID NO: 138 - RNA, 21 nt, synthetic construct
  source 1..21: mol_type = other RNA
tatcaggagagaatctattcg

SEQ ID NO: 139 - RNA, 21 nt, synthetic construct
  source 1..21: mol_type = other RNA
gcccaattaagtcctacttta

SEQ ID NO: 140 - RNA, 21 nt, synthetic construct
  source 1..21: mol_type = other RNA
taaagtaggacttaattgggc

SEQ ID NO: 141 - RNA, 21 nt, synthetic construct
  source 1..21: mol_type = other RNA
cgatcgctttctacactgtaa

SEQ ID NO: 142 - RNA, 21 nt, synthetic construct
  source 1..21: mol_type = other RNA
cgatcgctttctacactgtaa

SEQ ID NO: 143 - RNA, 21 nt, synthetic construct
  source 1..21: mol_type = other RNA
cctttctacactgtattacaa

SEQ ID NO: 144 - RNA, 21 nt, synthetic construct
  source 1..21: mol_type = other RNA
ttgtaatacagtgtagaaagg

SEQ ID NO: 145 - RNA, 19 nt, synthetic construct
  source 1..19: mol_type = other RNA
caaccaaccagtgaccata

SEQ ID NO: 146 - RNA, 21 nt, synthetic construct
  source 1..21: mol_type = other RNA
tggatggtcactggttggttg

SEQ ID NO: 147 - RNA, 21 nt, synthetic construct
  source 1..21: mol_type = other RNA
cccgaactgcagatcaccaaa

SEQ ID NO: 148 - RNA, 23 nt, synthetic construct
  source 1..23: mol_type = other RNA
tcattggtgatctgcagttcggg

SEQ ID NO: 149 - RNA, 19 nt, synthetic construct
  source 1..19: mol_type = other RNA
ctgccctgaactgcagata

SEQ ID NO: 150 - RNA, 21 nt, synthetic construct
  source 1..21: mol_type = other RNA
ttgatctgcagttcagggcag

SEQ ID NO: 151 - RNA, 21 nt, synthetic construct
  source 1..21: mol_type = other RNA
caagtctaccctgaactgcaa

SEQ ID NO: 152 - RNA, 21 nt, synthetic construct
  source 1..21: mol_type = other RNA
ttgcagttcagggtagacttg

SEQ ID NO: 153 - RNA, 19 nt, synthetic construct
  source 1..19: mol_type = other RNA
ggtctaccctgaactgcaa

SEQ ID NO: 154 - RNA, 21 nt, synthetic construct
  source 1..21: mol_type = other RNA
ttgcagttcagggtagacctc

SEQ ID NO: 155 - RNA, 19 nt, synthetic construct
  source 1..19: mol_type = other RNA
tagaagttctttgagcaga

SEQ ID NO: 156 - RNA, 21 nt, synthetic construct
  source 1..21: mol_type = other RNA
tatctgctcaaagaacttcta

SEQ ID NO: 157 - RNA, 21 nt, synthetic construct
  source 1..21: mol_type = other RNA
cccacaagttctttgagcaga

SEQ ID NO: 158 - RNA, 23 nt, synthetic construct
  source 1..23: mol_type = other RNA
tatctgctcaaagaacttgtggg

SEQ ID NO: 159 - RNA, 21 nt, synthetic construct
  source 1..21: mol_type = other RNA
aacaagtctaccctgaactga

SEQ ID NO: 160 - RNA, 23 nt, synthetic construct
  source 1..23: mol_type = other RNA
ttgcagttcagggtagacttgtt

SEQ ID NO: 161 - RNA, 19 nt, synthetic construct
  source 1..19: mol_type = other RNA
caccaatgtggtagaagca

SEQ ID NO: 162 - RNA, 21 nt, synthetic construct
  source 1..21: mol_type = other RNA
ttggcttctaccacattggtg

SEQ ID NO: 163 - RNA, 21 nt, synthetic construct
  source 1..21: mol_type = other RNA
gaggtctaccctgaactgcaa

SEQ ID NO: 164 - RNA, 21 nt, synthetic construct
  source 1..21: mol_type = other RNA
ttgcagttcagggtagacctc

SEQ ID NO: 165 - RNA, 21 nt, synthetic construct
  source 1..21: mol_type = other RNA
tacaagttctttgagcagata

SEQ ID NO: 166 - RNA, 23 nt, synthetic construct
  source 1..23: mol_type = other RNA
tatctgctcaaagaacttgtagg

SEQ ID NO: 167 - RNA, 19 nt, synthetic construct
  source 1..19: mol_type = other RNA
caagttctttgagcagata

SEQ ID NO: 168 - RNA, 21 nt, synthetic construct
  source 1..21: mol_type = other RNA
tatctgctcaaagaacttgta

SEQ ID NO: 169 - RNA, 21 nt, synthetic construct
  source 1..21: mol_type = other RNA
cctgtccaagatgcagcagaa

SEQ ID NO: 170 - RNA, 23 nt, synthetic construct
  source 1..23: mol_type = other RNA
ttctgctgcatcttggacaggtg

SEQ ID NO: 171 - RNA, 19 nt, synthetic construct
  source 1..19: mol_type = other RNA
tgtccaagatgcagcagaa

SEQ ID NO: 172 - RNA, 21 nt, synthetic construct
  source 1..21: mol_type = other RNA
tctgtccaagatgcagcagaa

SEQ ID NO: 173 - RNA, 21 nt, synthetic construct
  source 1..21: mol_type = other RNA
gaagtctaccctgaactgcaa

SEQ ID NO: 174 - RNA, 23 nt, synthetic construct
  source 1..23: mol_type = other RNA
ttgcagttcagggtagacttctt

SEQ ID NO: 175 - RNA, 19 nt, synthetic construct
  source 1..19: mol_type = other RNA
agtctaccctgaactgcaa

SEQ ID NO: 176 - RNA, 21 nt, synthetic construct
  source 1..21: mol_type = other RNA
ttgcagttcagggtagacttc

SEQ ID NO: 177 - RNA, 21 nt, synthetic construct
  source 1..21: mol_type = other RNA
cttacgctgagtacttcgatt

SEQ ID NO: 178 - RNA, 21 nt, synthetic construct
  source 1..21: mol_type = other RNA
tcgaagtactcagcgtaagtt

SEQ ID NO: 179 - DNA, 21 bp, synthetic construct
  source 1..21: mol_type = other DNA
ccttcccgtgaatggagagtt

SEQ ID NO: 180 - DNA, 19 bp, synthetic construct
  source 1..19: mol_type = other DNA
ctggtcgagtggtcagtcc

SEQ ID NO: 181 - DNA, 22 bp, synthetic construct
  source 1..22: mol_type = other DNA
cctggacgatctccagccgtgg

SEQ ID NO: 182 - DNA, 19 bp, synthetic construct
  source 1..19: mol_type = other DNA
gacagtcagccgcatcttc

SEQ ID NO: 183 - DNA, 19 bp, synthetic construct
  source 1..19: mol_type = other DNA
actccgaccttcaccttcc

SEQ ID NO: 184 - DNA, 20 bp, synthetic construct
  source 1..20: mol_type = other DNA
cgccagccgagccacatcgc

SEQ ID NO: 185 - protein, 19 aa, synthetic construct
TFFYGGSRGKRNNFKTEEY

SEQ ID NO: 186 - protein, 19 aa, synthetic construct
TFFYGGCRGKRNNFKTEEY